European Patent Application EP 4 527 395 A1, published March 26, 2025. Title: PHARMACEUTICAL COMPOSITION FOR PREVENTING AND TREATING AGE-RELATED DISEASES COMPRISING NEURAL STEM CELLS DERIVED FROM 3D HYPOTHALAMIC ORGANOID AND USE THEREOF. Applicant: 코아스템 켐온 주식회사. The sequence listing filed with the application follows.

SEQUENCE LISTING (14 sequences)

SEQ ID NO: 1 - DNA, 22 bp, synthetic construct
  misc_feature 1..22: note = NKX2-1 forward primer
  source 1..22: mol_type = other DNA
caggacaccatgaggaacagcg

SEQ ID NO: 2 - DNA, 22 bp, synthetic construct
  misc_feature 1..22: note = NKX2-1 reverse primer
  source 1..22: mol_type = other DNA
gccatgttcttgctcacgtccc

SEQ ID NO: 3 - DNA, 22 bp, synthetic construct
  misc_feature 1..22: note = RAX forward primer
  source 1..22: mol_type = other DNA
gcaaggtcaacctaccagaggt

SEQ ID NO: 4 - DNA, 22 bp, synthetic construct
  misc_feature 1..22: note = RAX reverse primer
  source 1..22: mol_type = other DNA
gcagcttcatggaggacacttc

SEQ ID NO: 5 - DNA, 22 bp, synthetic construct
  misc_feature 1..22: note = OTP forward primer
  source 1..22: mol_type = other DNA
agcttcgccaagactcactacc

SEQ ID NO: 6 - DNA, 22 bp, synthetic construct
  misc_feature 1..22: note = OTP reverse primer
  source 1..22: mol_type = other DNA
cacggaacacgttggtcgtctt

SEQ ID NO: 7 - DNA, 23 bp, synthetic construct
  misc_feature 1..23: note = ISL1 forward primer
  source 1..23: mol_type = other DNA
gcagagtgacatagatcagcctg

SEQ ID NO: 8 - DNA, 22 bp, synthetic construct
  misc_feature 1..22: note = ISL1 reverse primer
  source 1..22: mol_type = other DNA
gcctcaataggactggctacca

SEQ ID NO: 9 - DNA, 22 bp, synthetic construct
  misc_feature 1..22: note = SF-1 forward primer
  source 1..22: mol_type = other DNA
ccagaccttcatctccatcgtg

SEQ ID NO: 10 - DNA, 22 bp, synthetic construct
  misc_feature 1..22: note = SF-1 reverse primer
  source 1..22: mol_type = other DNA
tggcggtagatgtggtcgaaca

SEQ ID NO: 11 - DNA, 23 bp, synthetic construct
  misc_feature 1..23: note = EN1 forward primer
  source 1..23: mol_type = other DNA
gcaacccggctatcctacttatg

SEQ ID NO: 12 - DNA, 21 bp, synthetic construct
  misc_feature 1..21: note = EN1 reverse primer
  source 1..21: mol_type = other DNA
atgtagcggtttgcctggaac

SEQ ID NO: 13 - DNA, 20 bp, synthetic construct
  misc_feature 1..20: note = ACTB forward primer
  source 1..20: mol_type = other DNA
gtgacagcagtcggttggag

SEQ ID NO: 14 - DNA, 23 bp, synthetic construct
  misc_feature 1..23: note = ACTB reversed primer
  source 1..23: mol_type = other DNA
aacaacgcatctcatatttggaa